European Patent Specification EP 3 291 843 B1, published March 22, 2023. Title: Modified UBE3A Gene for a Gene Therapy Approach for Angelman Syndrome. Applicant: University of South Florida. The sequence listing filed with the application follows.

SEQUENCE LISTING (15 sequences)

SEQ ID NO: 1 - DNA, 2550 bp, Mus musculus
atgaagcgagcagctgcaaagcatctaatagaacgctactaccatcagttaactgagggctgtggaaatgaggcctgcacgaatgagttttgtgcttcctgtccaacttttcttcgtatggataacaatgcagcagctattaaagcccttgagctttataaaattaatgcaaaactctgtgatcctcatccctccaagaaaggagcaagctcagcttaccttgagaactcaaaaggtgcatctaacaactcagagataaaaatgaacaagaaggaaggaaaagattttaaagatgtgatttacctaactgaagagaaagtatatgaaatttatgaattttgtagagagagtgaggattattcccctttaattcgtgtaattggaagaatattttctagtgctgaggcactggttctgagctttcggaaagtcaaacagcacacaaaggaggaattgaaatctcttcaagaaaaggatgaagacaaggatgaagatgaaaaggaaaaagctgcatgttctgctgctgctatggaagaagactcagaagcatcttcttcaaggatgggtgatagttcacagggagacaacaatgtacaaaaattaggtcctgatgatgtgactgtggatattgatgctattagaagggtctacagcagtttgctcgctaatgaaaaattagaaactgccttcctgaatgcacttgtatatctgtcacctaacgtggaatgtgatttgacatatcataatgtgtatactcgagatcctaattatctcaatttgttcattattgtaatggagaatagtaatctccacagtcctgaatatctggaaatggcgttgccattattttgcaaagctatgtgtaagctaccccttgaagctcaaggaaaactgattaggctgtggtctaaatacagtgctgaccagattcggagaatgatggaaacatttcagcaacttattacctacaaagtcataagcaatgaatttaatagccgaaatctagtgaatgatgatgatgccattgttgctgcttcaaagtgtttgaaaatggtttactatgcaaatgtagtgggaggggatgtggacacaaatcataatgaggaagatgatgaagaacccatacctgagtccagcgaattaacacttcaggagcttctgggagatgaaagaagaaataagaaaggtcctcgagtggatccactagaaaccgaacttggcgttaaaactctagactgtcgaaaaccacttatctcctttgaagaattcattaatgaaccactgaatgatgttctagaaatggacaaagattatacctttttcaaagttgaaacagagaacaaattctcttttatgacatgtccctttatattgaatgctgtcacaaagaatctgggattatattatgacaatagaattcgcatgtacagtgaaagaagaatcactgttctttacagcctagttcaaggacagcagttgaatccgtatttgagactcaaagtcagacgtgaccatattatagatgatgcactggtccggctagagatgattgctatggaaaatcctgcagacttgaagaagcagttgtatgtggaatttgaaggagaacaaggagtaatgagggaggcgtttccaaagagttttttcagttgggttgtggaggaaatttttaatccaaatattggtatgttcacatatgatgaagctacgaaattattttggtttaatccatcttcttttgaaactgagggtcaggtttactctgattggcatatcctgggtctggctatttacaataattgtatactggatgtccattttcccatggttgtatacaggaagctaatggggaaaaaaggaacctttcgtgacttgggagactctcacccagttttatatcagagtttaaaggatttattggaatatgaagggagtgtggaagatgatatgatgatcactttccagatatcacagacagatctttttggtaacccaatgatgtatgatctaaaagaaaatggtgataaaattccaattacaaatgaaaacaggaaggaatttgtcaatctctattcagactacattctcaataaatctgtagaaaaacaattcaaggcatttcgcagaggttttcatatggtgactaatgaatcgcccttaaaatacttattcagaccagaagaaattgaattgcttatatgtggaagccggaatctagatttccaggcactagaagaaactacagagtatgacggtggctatacgagggaatctgttgtgattagggagttctgggaaattgttcattcgtttacagatgaacagaaaagactctttctgcagtttacaacaggcacagacagagcacctgttggaggactaggaaaattgaagatgattatagccaaaaatggcccagacacagaaaggttacctacatctcatacttgctttaatgtccttttacttccggaatattcaagcaaagaaaaacttaaagagagattgttgaaggccatcacatatgccaaaggatttggcatgctgtaa

SEQ ID NO: 2 - DNA, 78 bp, Mus musculus
atggccctgttggtgcacttcctacccctgctggccctgcttgccctctgggagcccaaacccacccaggcttttgtc

SEQ ID NO: 3 - protein, 26 aa, Mus musculus
MALLVHFLPLLALLALWEPKPTQAFV

SEQ ID NO: 4 - DNA, 33 bp, Human immunodefiency virus
tacggcagaaagaagaggaggcagagaaggaga

SEQ ID NO: 5 - protein, 11 aa, Human immunodeficiency virus
YGRKKRRQRRR

SEQ ID NO: 6 - DNA, 10893 bp, Homo sapiens
  misc_feature (122)..(122): n is a, c, g, or t
  misc_feature (340)..(340): n is a, c, g, or t
  misc_feature (1145)..(1145): n is a, c, g, or t
  misc_feature (1180)..(1180): n is a, c, g, or t
  misc_feature (1257)..(1257): n is a, c, g, or t
  misc_feature (5410)..(5410): n is a, c, g, or t
  misc_feature (7624)..(7624): n is a, c, g, or t
  misc_feature (7644)..(7644): n is a, c, g, or t
  misc_feature (7647)..(7647): n is a, c, g, or t
  misc_feature (7741)..(7741): n is a, c, g, or t
  misc_feature (7836)..(7836): n is a, c, g, or t
ggagtagtttactgagccactaatctaaagtttaatactgtgagtgaataccagtgagtacctttgttaatgtggataaccaatacttggctataggaagttttttagttgtgtgttttatnacacgtatttgactttgtgaataattatggcttataatggcttgtctgttggtatctatgtatagcgtttacagtttcctttaaaaaacatgcattgagttttttaatagtccaacccttaaaataaatgtgttgtatggccacctgatctgaccactttctttcatgttgacatctttaattttaaaactgttttatttagtgcttaaatcttgttnacaaaattgtcttcctaagtaatatgtctacctttttttttggaatatggaatattttgctaactgtttctcaattgcattttacagatcaggagaacctcagtctgacgacattgaagctagccgaatgtaagtgtaacttggttgagactgtggttcttattttgagttgccctagactgctttaaattacgtcacattatttggaaataatttctggttaaaagaaaggaatcatttagcagtaaatgggagataggaacatacctactttttttcctatcagataactctaaacctcggtaacagtttactaggtttctactactagatagataaatgcacacgcctaaattcttagtctttttgcttccctggtagcagttgtagggaaatagggaggttgaggaaagagtttaacagtctcaacgcctaccatatttaaggcatcaagtactatgttatagatacagagatgcgtaataattagttttcaccctacagaaatttatattatactcaagagtgaaagatgcagaagcaaataatttcagtcactgaggtagaatggtatccaaaatacaatagtaacatgaaggagtactggagtaccaggtatgcaataggaatctagtgtagatggcagggaagtaagagtggccaggaaatgctaagttcagtcttgaaatgtgactgggaatcaggcagctatcaactataagtcaaatgtttacaagctgttaaaaatgaaatactgattatgtaaaagaaaaccggattgatgctttaaatagactcattttcntaatgctaatttttaaaatgatagaatcctacaantcttagctgtaaaccttgtgatttttcagctgttgtactaaacaacttaagcacatataccatcagacaagcccccntccccccttttaaaccaaaggaatgtatactctgttaatacagtcagtaagcattgacattctttatcataatatcctagaaaatatttattaactatttcactagtcaggagttgtggtaaatagtgcatctccattttctacttctcatcttcatacacaggttaatcacttcagtgcttgactaacttttgccttgatgatatgttgagctttgtacttgagagctgtactaatcactgtgcttattgtttgaatgtttggtacaggaagcgagcagctgcaaagcatctaatagaacgctactaccaccagttaactgagggctgtggaaatgaagcctgcacgaatgagttttgtgcttcctgtccaacttttcttcgtatggataataatgcagcagctattaaagccctcgagctttataagattaatgcaaaactctgtgatcctcatccctccaagaaaggagcaagctcagcttaccttgagaactcgaaaggtgcccccaacaactcctgctctgagataaaaatgaacaagaaaggcgctagaattgattttaaaggtaagatgttttattttcaattgagaattgttgcctgaaaaccatgtgggagatttaaatgtattagtttttatttgttttttcttctgtgacataaagacattttgatatcgtagaaccaattttttattgtggtaacggacaggaataataactacattttacaggtctaatcattgctaattagaagcagatcatatgccaaaagttcatttgttaatagattgatttgaactttttaaaattcttaggaaaaatgtattaagtggtagtgaatctccaaaactatttaagagctgtattatgattaatcagtacatgacatattggttcatatttataattaaagctatacattaatagatatcttgattataaagaaagtttaaactcatgatcttattaagagttatacattgttgaaagaatgtaaaagcatgggtgaggtcattggtataggtaggtagttcattgaaaaaaataggtaagcattaaattttgtttgctgaatctaagtattagatactttaagagttgtatatcataaatgatattgagcctagaatgtttggctgttttacttttagaactttttgcaacagagtaaacatacatattatgaaaataaatgttctcttttttcctctgattttctagatgtgacttacttaacagaagagaaggtatatgaaattcttgaattatgtagagaaagagaggattattcccctttaatccgtgttattggaagagttttttctagtgctgaggcattggtacagagcttccggaaagttaaacaacacaccaaggaagaactgaaatctcttcaagcaaaagatgaagacaaagatgaagatgaaaaggaaaaagctgcatgttctgctgctgctatggaagaagactcagaagcatcttcctcaaggataggtgatagctcacagggagacaacaatttgcaaaaattaggccctgatgatgtgtctgtggatattgatgccattagaagggtctacaccagattgctctctaatgaaaaaattgaaactgcctttctcaatgcacttgtatatttgtcacctaacgtggaatgtgacttgacgtatcacaatgtatactctcgagatcctaattatctgaatttgttcattatcgtaatggagaatagaaatctccacagtcctgaatatctggaaatggctttgccattattttgcaaagcgatgagcaagctaccccttgcagcccaaggaaaactgatcagactgtggtctaaatacaatgcagaccagattcggagaatgatggagacatttcagcaacttattacttataaagtcataagcaatgaatttaacagtcgaaatctagtgaatgatgatgatgccattgttgctgcttcgaagtgcttgaaaatggtttactatgcaaatgtagtgggaggggaagtggacacaaatcacaatgaagaagatgatgaagagcccatccctgagtccagcgagctgacacttcaggaacttttgggagaagaaagaagaaacaagaaaggtcctcgagtggaccccctggaaactgaacttggtgttaaaaccctggattgtcgaaaaccacttatcccttttgaagagtttattaatgaaccactgaatgaggttctagaaatggataaagattatacttttttcaaagtagaaacagagaacaaattctcttttatgacatgtccctttatattgaatgctgtcacaaagaatttgggattatattatgacaatagaattcgcatgtacagtgaacgaagaatcactgttctctacagcttagttcaaggacagcagttgaatccatatttgagactcaaagttagacgtgaccatatcatagatgatgcacttgtccgggtaagttgggctgctagattaaaaacctaataatggggatatcatgatacagttcagtgaattcattttaaaagtgactgaaaaaaatgataccatatagcataggaacacatggacatttctgatcttatataagtattatacttttgttgttcctgtgcaagtttatagatgtgttctacaaagtatcggttgtattatataatggtcatgctatctttgaaaaagaatgggttttctaaatcttgaaaactaaatccaaagtttctttcattcagaagagaatagagtgttggacaaagaccagaacaagagaaatgtggagatacccaataataagtgtggatgtgcagtcttgaactgggagtaatggtacagtaaaaccataccataaaattataggtagtgtccaaaaaattccatcgtgtaaaattcagagttgcattattgtggacttgaagaagcagttgtatgtgggacggtatcgataagcttgatatcgaattcctgcagcccgggggatccactagtgtggtaattaatactaagtcttactgtgagagaccataaactgctttagtattcagtgtatttttcttaattgaaatatttaacttatgacttagtagatactaagacttaacccttgagtttctattctaataaaggactactaatgaacaattttgaggttagacctctactccattgtttttgctgaaatgatttagctgcttttccatgtcctgtgtagtccagacttaacacacaagtaataaaatcttaattaattgtatgttaatttcataacaaatcagtaaagttagctttttactatgctagtgtctgttttgtgtctgtctttttgattatctttaagactgaatctttgtcttcactggctttttatcagtttgctttctgtttccatttacatacaaaaagtcaaaaatttgtatttgtttcctaatcctactccttgtttttattttgtttttttcctgatactagcaatcatcttcttttcatgtttatcttttcaatcactagctagagatgatcgctatggaaaatcctgcagacttgaagaagcagttgtatgtggaatttgaaggagaacaaggagttgatgagggaggtgtttccaaagaattttttcagctggttgtggaggaaatcttcaatccagatattggtaaatacattagtaatgtgattatggtgtcgtatcatcttttgagttagttatttgtttatcttactttgtaaatattttcagctatgaagagcagcaaaagaaggatttggtatggattacccagaatcacacatcatgactgaatttgtaggttttaggaactgatttgtatcactaatttattcaaattcttttatttcttagaaggaatattctaatgaaggaaattatctctttggtaaactgaattgaaagcactttagaatggtatattggaacagttggagggatttctttgctttttgttgtctaaaaccatcatcaaactcacggttttcctgacctgtgaacttcaaagaacaatggtttgaagagtattgagagactgtctcacaagtatgtcatgctcaaagttcagaaacactagctgatatcacattaattaggtttatttgctataagatttcttggggcttaatatangtagtgttcccccaaactttttgaactccagaactcttttctgccctaacagtagctactcaggagctgaggcaggagaattgtttgaacctaggaggcagaggttgcagtgagctgagatcgtgccactccagcccacccctgggtaacagagcgagactccatctcaaagaaaaaaatgaaaaattgttttcaaaaatagtacgtgtggtacagatataagtaattatatttttataaatgaaacactttggaaatgtagccattttttgtttttttatgtttatttttcagctatgggtggataaagcatgaatataacttttcttatgtgttagtagaaaattagaaagcttgaatttaattaacgtatttttctacccgatgccaccaaattacttactactttattcctttggcttcataaaattacatatcaccattcaccccaatttatagcagatatatgtggacattgttttctcaagtgctaatataatagaaatcaatgttgcatgcctaattacatatattttaaatgttttatatgcataattattttaagtttatatttgtattattcatcagtccttaataaaatacaaaagtaatgtatttttaaaaatcatttcttataggtatgttcacatacgatgaatctacaaaattgttttggtttaatccatcttcttttgaaactgagggtcagtttactctgattggcatagtactgggtctggctatttacaataactgtatactggatgtacattttcccatggttgtctacaggaagctaatggggaaaaaaggaacttttcgtgacttgggagactctcacccagtaagttctttgtcatttttttaattcagtctcttagattttatttaaatgcaaaaatttaatttatgtcaaaattttaaagtttttgtttagaatctttgttgatactcttatcaataagataaaaatgttttaatctgaccgaagtaccagaaacacttaaaaactcaaagggggacatttttatatattgctgtcagcacgaagctttcgtaagattgatttcatagagaagtgtttctaaacattttgtttgtgttttagtgaaatcttaagagataggtaaaaatcagagtagccctggctaagggtcttggtagttacaacgagtgtgcctgctcctaccacccccacccccaccttgagacaccacagaatttctcatagagcacagtgtgaattctattgctaaattggtggtatggggtttctcagcagagaatgggacatcacagtgactgacaatctttcttttataggttggaaactatttgggggactggagggatactgtctacactttttacaatttttattgataagatttttgttgtcttctaagaagagtgatataaattatttgttgtattttgtagttctatggtggcctcaatttaccatttctggttgctaggttctatatcagagtttaaaagatttattggagtatgaagggaatgtggaagatgacatgatgatcactttccagatatcacagacagatctttttggtaacccaatgatgtatgatctaaaggaaaatggtgataaaattccaattacaaatgaaaacaggaaggtaataaatgtttttatgtcacattttgtctcttcattaacactttcaaagcatgtatgcttataatttttaaagaagtatctaatatagtctgtacaaaaaaaaaacaagtaactaagtttatgtaaatgctagagtccacttttctaaatcttggatataagttggtatgaaagcacacagttgggcactaaagccccttttagagaaagaggacatgaagcaggagatagttaatagctaagtgtggttgtagtataaagcaagaagcagggtgtttcttgtattaagctgtaagcaggaacctcatgattaaggtctttatcacagaacaaataaaaattacatttaatttacacatgtatatcctgtttgtgataaaaatacatttctgaaaagtatactttacgtcagatttgggttctattgactaaaatgtgttcatcgggaatgggaataacccagaacataacaagcaaaaaattatgacaaatatatagtatacctttaagaaacatgtttatattgatataattttttgattaaatattatacacactaagggtacaangcacattttccttttatganttngatacagtagtttatgtgtcagtcagatacttccacatttttgctgaactggatacagtaagcagcttaccaaatattctatggtagaaaactnggacttcctggtttgcttaaatcaaatatattgtactctcttaaaacggttggcatttataaatagatggatacatggtttaaatgtgtctgttnacatacctagttgagagaacctaaagaattttctgcgtctccagcatttatattcagttctgtttaatacattatcgaaattgacatttataagtatgacagttttgtgtatatggccttttcatagcttaatattggctgtaacagagaattgtgaaattgtaagaagtagttttctttgtaggtgtaaaattgaatttttaagaatattcttgacagttttatgtatatggccttttcatagcttaatattggctataacagagaattgtgaaattgttaagaagtaggtgtaaaattgaatttttaagaatattcttgaatgtttttttcttggaaaaattaaaaagctatgcagcccaataacttgtgttttgtttgcatagcatattataagaagttcttgtgattaatgttttctacaggaatttgtcaatctttattctgactacattctcaataaatcagtagaaaaacagttcaaggcttttcggagaggttttcatatggtgaccaatgaatctcccttaaagtacttattcagaccagaagaaattgaattgcttatatgtggaagccgggtaagaaagcaggtgtctgcaaaaagtcatgtatcgatttattgtttgtaatgatacagtagtatagcagataactaagacatattttcttgaatttgcagaatctagatttccaagcactagaagaaactacagaatatgacggtggctataccagggactctgttctgattaggtgaggtacttagttcttcagaggaagatttgattcaccaaaggggtgtgtgattttgcttcagacctttatctctaggtactaattcccaaataagcaaactcacaaattgtcatctatatacttagatttgtatttgtaatataatcaccatttttcagagctaatcttgtgatttatttcatgaatgaagtgttgttatatataagtctcatgtaatctcctgcatttggcgtatggattatctagtattcctcactggttagagtatgcttactgctggttagaagataattaaaataaggctaccatgtctgcaatttttcctttcttttgaactctgcatttgtgaactgttacatggcttcccaggatcaagcactttttgagtgaaatggtagtcttttatttaattcttaagataatatgtccagatacatactagtatttccattttacaccctaaaaaactaagccctgaattctcacagaaagatgtagaggttcccagttctatctgcttttaaacaaatgcccttactactctactgtctacttctgtgtactacatcatcgtatgtagttgtttgcatttgggccagttggttggggcaggggtctttttttcttttgtcccttaatctgtatcactttttcctcccaaagttgagttaaaggatgagtagaccaggagaataaaggagaaaggataaataaaatatatacccaaaggcacctggagttaatttttccaaatattcatttcagtctttttcaattcataggattttgtcttttgctcattactgactgcataatgtgattataccatagtttaaatagtcacttcctgttactacacacttgggttttctcaattttttactattgtagtactaatattttactatattgtaatctaatccaaatttttacgtattcagagctgttcaggataaatttgcttggaaatttttaaatcaccagaagtgatactatcctgataattaacttccaagttgtctcttaatatagttttaatgcaaatcataagcttatgttagtaccagtcataatgaatgccaaactgaaaccagtattgtattttttctcattagggagttctgggaaatcgttcattcatttacagatgaacagaaaagactcttcttgcagtttacaacgggcacagacagagcacctgtgggaggactaggaaaattaaagatgattatagccaaaaatggcccagacacagaaaggtaggtaattattaacttgtgactgtatacctaccgaaaaccttgcattcctcgtcacatacatatgaactgtctttatagtttctgagcacattcgtgattttatatacaaatccccaaatcatattagacaattgagaaaatactttgctgtcattgtgtgaggaaacttttaagaaattgccctagttaaaaattattatggggctcacattggtttggaatcaaattagtgtgattcatttacttttttgattcccagcttgttaattgaaagccatataacatgatcatctatttagaatggttacattgaggctcggaagattatcatttgattgtgctagaatcctgttatcaaatcattttcttagtcatattgccagcagtgtttctaataagcatttaagagcacacactttgcagtcttgtaaaacaggtttgagtattttctccaccttagaggaagttacttgacttctcagtgacctaacctctaaagtgcatttactgatgtcctctctgtggttttgttgtggaaagatttagttaaatgaactgtaagaattcagtacctaaaatggtatctgttatgtagtaaaaactcaatggatacagtatcttatcatcgtcactagctttgagtaatttataggataaaggcaacttggtagttacacaacaaaaagtttatgatttgcattaatgtatagtttgcattgcagaccgtctcaactatatacaatctaaaaataggagcatttaattctaagtgtatttcccatgacttacagttttcctgtttttttccccttttctctatttaggttacctacatctcatacttgctttaatgtgcttttacttccggaatactcaagcaaagaaaaacttaaagagagattgttgaaggccatcacgtatgccaaaggatttggcatgctgtaaaacaaaacaaaacaaaataaaacaaaaaaaaggaaggaaaaaaaaagaaaaaatttaaaaaattttaaaaatataacgagggataaatttt

SEQ ID NO: 7 - protein, 852 aa, Homo sapiens
MKRAAAKHLIERYYHQLTEGCGNEACTNEFCASCPTFLRMDNNAAAIKALELYKINAKLCDPHPSKKGASSAYLENSKGAPNNSCSEIKMNKKGARIDFKDVTYLTEEKVYEILELCREREDYSPLIRVIGRVFSSAEALVQSFRKVKQHTKEELKSLQAKDEDKDEDEKEKAACSAAAMEEDSEASSSRIGDSSQGDNNLQKLGPDDVSVDIDAIRRVYTRLLSNEKIETAFLNALVYLSPNVECDLTYHNVYSRDPNYLNLFIIVMENRNLHSPEYLEMALPLFCKAMSKLPLAAQGKLIRLWSKYNADQIRRMMETFQQLITYKVISNEFNSRNLVNDDDAIVAASKCLKMVYYANVVGGEVDTNHNEEDDEEPIPESSELTLQELLGEERRNKKGPRVDPLETELGVKTLDCRKPLIPFEEFINEPLNEVLEMDKDYTFFKVETENKFSFMTCPFILNAVTKNLGLYYDNRIRMYSERRITVLYSLVQGQQLNPYLRLKVRRDHIIDDALVRLEMIAMENPADLKKQLYVEFEGEQGVDEGGVSKEFFQLVVEEIFNPDIGMFTYDESTKLFWFNPSSFETEGQFTLIGIVLGLAIYNNCILDVHFPMVVYRKLMGKKGTFRDLGDSHPVLYQSLKDLLEYEGNVEDDMMITFQISQTDLFGNPMMYDLKENGDKIPITNENRKEFVNLYSDYILNKSVEKQFKAFRRGFHMVTNESPLKYLFRPEEIELLICGSRNLDFQALEETTEYDGGYTRDSVLIREFWEIVHSFTDEQKRLFLQFTTGTDRAPVGGLGKLKMIIAKNGPDTERLPTSHTCFNVLLLPEYSSKEKLKERLLKAITYAKGFGML

SEQ ID NO: 8 - DNA, 57 bp, Homo sapiens
atgaagttatgggatgtcgtggctgtctgcctggtgctgctccacaccgcgtccgcc

SEQ ID NO: 9 - DNA, 72 bp, Homo sapiens
atggccctgtggatgcgcctcctgcccctgctggcgctgctggccctctggggacctgacccagccgcagcc

SEQ ID NO: 10 - DNA, 60 bp, Homo sapiens
atggagacagacacactcctgctatgggtactgctgctctgggttccaggttccactggt

SEQ ID NO: 11 - protein, 11 aa, human immunodeficiency virus
YARKAARQARA

SEQ ID NO: 12 - DNA, 2767 bp, Homo sapiens
acagtatgacatctgatgctggagggtcgcactttcacaaatgagtcagctggtacatggggttatcatcaatttttagctcttctgtctgggagatacaagtttggaagcaatcttggggtacttacccacaaggctggtggagaccagatcaggagaacctcagtctgacgacattgaagctagccgaatgaagcgagcagctgcaaagcatctaatagaacgctactaccaccagttaactgagggctgtggaaatgaagcctgcacgaatgagttttgtgcttcctgtccaacttttcttcgtatggataataatgcagcagctattaaagccctcgagctttataagattaatgcaaaactctgtgatcctcatccctccaagaaaggagcaagctcagcttaccttgagaactcgaaaggtgcccccaacaactcctgctctgagataaaaatgaacaagaaaggcgctagaattgattttaaagatgtgacttacttaacagaagagaaggtatatgaaattcttgaattatgtagagaaagagaggattattcccctttaatccgtgttattggaagagttttttctagtgctgaggcattggtacagagcttccggaaagttaaacaacacaccaaggaagaactgaaatctcttcaagcaaaagatgaagacaaagatgaggatgaaaaggaaaaagctgcatgttctgctgctgctatggaagaagactcagaagcatcttcctcaaggataggtgatagctcacagggagacaacaatttgcaaaaattaggccctgatgatgtgtctgtggatattgatgccattagaagggtctacaccagattgctctctaatgaaaaaattgaaactgcctttctcaatgcacttgtatatttgtcacctaacgtggaatgtgacttgacgtatcacaatgtatactctcgagatcctaattatctgaatttgttcattatcgtaatggagaatagaaatctccacagtcctgaatatctggaaatggctttgccattattttgcaaagcgatgagcaagctaccccttgcagcccaaggaaaactgatcagactgtggtctaaatacaatgcagaccagattcggagaatgatggagacatttcagcaacttattacttataaagtcataagcaatgaatttaacagtcgaaatctagtgaatgatgatgatgccattgttgctgcttcgaagtgcttgaaaatggtttactatgcaaatgtagtgggaggggaagtggacacaaatcacaatgaagaagatgatgaagagcccatccctgagtccagcgagctgacacttcaggaacttttgggagaagaaagaagaaacaagaaaggtcctcgagtggaccccctggaaactgaacttggtgttaaaaccctggattgtcgaaaaccacttatcccttttgaagagtttattaatgaaccactgaatgaggttctagaaatggataaagattatacttttttcaaagtagaaacagagaacaaattctcttttatgacatgtccctttatattgaatgctgtcacaaagaatttgggattatattatgacaatagaattcgcatgtacagtgaacgaagaatcactgttctctacagcttagttcaaggacagcagttgaatccatatttgagactcaaagttagacgtgaccatatcatagatgatgcacttgtccggctagagatgatcgctatggaaaatcctgcagacttgaagaagcagttgtatgtggaatttgaaggagaacaaggagttgatgagggaggtgtttccaaagaattttttcagctggttgtggaggaaatcttcaatccagatattggtatgttcacatacgatgaatctacaaaattgttttggtttaatccatcttcttttgaaactgagggtcagtttactctgattggcatagtactgggtctggctatttacaataactgtatactggatgtacattttcccatggttgtctacaggaagctaatggggaaaaaaggaacttttcgtgacttgggagactctcacccagttctatatcagagtttaaaagatttattggagtatgaagggaatgtggaagatgacatgatgatcactttccagatatcacagacagatctttttggtaacccaatgatgtatgatctaaaggaaaatggtgataaaattccaattacaaatgaaaacaggaaggaatttgtcaatctttattctgactacattctcaataaatcagtagaaaaacagttcaaggcttttcggagaggttttcatatggtgaccaatgaatctcccttaaagtacttattcagaccagaagaaattgaattgcttatatgtggaagccggaatctagatttccaagcactagaagaaactacagaatatgacggtggctataccagggactctgttctgattagggagttctgggaaatcgttcattcatttacagatgaacagaaaagactcttcttgcagtttacaacgggcacagacagagcacctgtgggaggactaggaaaattaaagatgattatagccaaaaatggcccagacacagaaaggttacctacatctcatacttgctttaatgtgcttttacttccggaatactcaagcaaagaaaaacttaaagagagattgttgaaggccatcacgtatgccaaaggatttggcatgctgtaaaacaaaacaaaacaaaat

SEQ ID NO: 13 - DNA, 5276 bp, Homo sapiens
agccagtcctcccgtcttgcgccgcggccgcgagatccgtgtgtctcccaagatggtggcgctgggctcggggtgactacaggagacgacggggccttttcccttcgccaggacccgacacaccaggcttcgctcgctcgcgcacccctccgccgcgtagccatccgccagcgcgggcgcccgccatccgccgcctacttacgcttcacctctgccgacccggcgcgctcggctgcgggcggcggcgcctccttcggctcctcctcggaatagctcgcggcctgtagcccctggcaggagggcccctcagccccccggtgtggacaggcagcggcggctggcgacgaacgccgggatttcggcggccccggcgctccctttcccggcctcgttttccggataaggaagcgcgggtcccgcatgagccccggcggtggcggcagcgaaagagaacgaggcggtggcgggcggaggcggcgggcgagggcgactacgaccagtgaggcggccgccgcagcccaggcgcgggggcgacgacaggttaaaaatctgtaagagcctgattttagaattcaccagctcctcagaagtttggcgaaatatgagttattaagcctacgctcagatcaaggtagcagctagactggtgtgacaacctgtttttaatcagtgactcaaagctgtgatcaccctgatgtcaccgaatggccacagcttgtaaaagagagttacagtggaggtaaaaggagtggcttgcaggatggagaagctgcaccagtgttattggaaatcaggagaacctcagtctgacgacattgaagctagccgaatgaagcgagcagctgcaaagcatctaatagaacgctactaccaccagttaactgagggctgtggaaatgaagcctgcacgaatgagttttgtgcttcctgtccaacttttcttcgtatggataataatgcagcagctattaaagccctcgagctttataagattaatgcaaaactctgtgatcctcatccctccaagaaaggagcaagctcagcttaccttgagaactcgaaaggtgcccccaacaactcctgctctgagataaaaatgaacaagaaaggcgctagaattgattttaaagatgtgacttacttaacagaagagaaggtatatgaaattcttgaattatgtagagaaagagaggattattcccctttaatccgtgttattggaagagttttttctagtgctgaggcattggtacagagcttccggaaagttaaacaacacaccaaggaagaactgaaatctcttcaagcaaaagatgaagacaaagatgaagatgaaaaggaaaaagctgcatgttctgctgctgctatggaagaagactcagaagcatcttcctcaaggataggtgatagctcacagggagacaacaatttgcaaaaattaggccctgatgatgtgtctgtggatattgatgccattagaagggtctacaccagattgctctctaatgaaaaaattgaaactgcctttctcaatgcacttgtatatttgtcacctaacgtggaatgtgacttgacgtatcacaatgtatactctcgagatcctaattatctgaatttgttcattatcgtaatggagaatagaaatctccacagtcctgaatatctggaaatggctttgccattattttgcaaagcgatgagcaagctaccccttgcagcccaaggaaaactgatcagactgtggtctaaatacaatgcagaccagattcggagaatgatggagacatttcagcaacttattacttataaagtcataagcaatgaatttaacagtcgaaatctagtgaatgatgatgatgccattgttgctgcttcgaagtgcttgaaaatggtttactatgcaaatgtagtgggaggggaagtggacacaaatcacaatgaagaagatgatgaagagcccatccctgagtccagcgagctgacacttcaggaacttttgggagaagaaagaagaaacaagaaaggtcctcgagtggaccccctggaaactgaacttggtgttaaaaccctggattgtcgaaaaccacttatcccttttgaagagtttattaatgaaccactgaatgaggttctagaaatggataaagattatacttttttcaaagtagaaacagagaacaaattctcttttatgacatgtccctttatattgaatgctgtcacaaagaatttgggattatattatgacaatagaattcgcatgtacagtgaacgaagaatcactgttctctacagcttagttcaaggacagcagttgaatccatatttgagactcaaagttagacgtgaccatatcatagatgatgcacttgtccggctagagatgatcgctatggaaaatcctgcagacttgaagaagcagttgtatgtggaatttgaaggagaacaaggagttgatgagggaggtgtttccaaagaattttttcagctggttgtggaggaaatcttcaatccagatattggtatgttcacatacgatgaatctacaaaattgttttggtttaatccatcttcttttgaaactgagggtcagtttactctgattggcatagtactgggtctggctatttacaataactgtatactggatgtacattttcccatggttgtctacaggaagctaatggggaaaaaaggaacttttcgtgacttgggagactctcacccagttctatatcagagtttaaaagatttattggagtatgaagggaatgtggaagatgacatgatgatcactttccagatatcacagacagatctttttggtaacccaatgatgtatgatctaaaggaaaatggtgataaaattccaattacaaatgaaaacaggaaggaatttgtcaatctttattctgactacattctcaataaatcagtagaaaaacagttcaaggcttttcggagaggttttcatatggtgaccaatgaatctcccttaaagtacttattcagaccagaagaaattgaattgcttatatgtggaagccggaatctagatttccaagcactagaagaaactacagaatatgacggtggctataccagggactctgttctgattagggagttctgggaaatcgttcattcatttacagatgaacagaaaagactcttcttgcagtttacaacgggcacagacagagcacctgtgggaggactaggaaaattaaagatgattatagccaaaaatggcccagacacagaaaggttacctacatctcatacttgctttaatgtgcttttacttccggaatactcaagcaaagaaaaacttaaagagagattgttgaaggccatcacgtatgccaaaggatttggcatgctgtaaaacaaaacaaaacaaaataaaacaaaaaaaaggaaggaaaaaaaaagaaaaaatttaaaaaattttaaaaatataacgagggataaatttttggtggtgatagtgtcccagtacaaaaaggctgtaagatagtcaaccacagtagtcacctatgtctgtgcctcccttctttattggggacatgtgggctggaacagcagatttcagctacatatatgaacaaatcctttattattattataattatttttttgcgtgaaagtgttacatattctttcacttgtatgtacagagaggtttttctgaatatttattttaagggttaaatcacttttgcttgtgtttattactgcttgaggttgagccttttgagtatttaaaaaatatataccaacagaactactctcccaaggaaaatattgccaccatttgtagaccacgtaaccttcaagtatgtgctacttttttgtccctgtatctaactcaaatcaggaactgtattttttttaatgatttgcttttgaaacttgaagtcttgaaaacagtgtgatgcaattactgctgttctagcccccaaagagttttctgtgcaaaatcttgagaatcaatcaataaagaaagatggaaggaagggagaaattggaatgttttaactgcagccctcagaactttagtaacagcacaacaaattaaaaacaaaaacaactcatgccacagtatgtcgtcttcatgtgtcttgcaatgaactgtttcagtagccaatcctctttcttagtatatgaaaggacagggatttttgttcttgttgttctcgttgttgttttaagtttactggggaaagtgcatttggccaaatgaaatggtagtcaagcctattgcaacaaagttaggaagtttgttgtttgtttattataaacaaaaagcatgtgaaagtgcacttaagatagagtttttattaattacttacttattacctagattttaaatagacaatccaaagtctccccttcgtgttgccatcatcttgttgaatcagccattttatcgaggcacgtgatcagtgttgcaacataatgaaaaagatggctactgtgccttgtgttacttaatcatacagtaagctgacctggaaatgaatgaaactattactcctaagaattacattgtatagccccacagattaaatttaattaattaattcaaaacatgttaaacgttactttcatgtactatggaaaagtacaagtaggtttacattactgatttccagaagtaagtagtttcccctttcctagtcttctgtgtatgtgatgttgttaatttcttttattgcattataaaataaaaggattatgtatttttaactaaggtgagacattgatatatccttttgctacaagctatagctaatgtgctgagcttgtgccttggtgattgattgattgattgactgattgttttaactgattactgtagatcaacctgatgatttgtttgtttgaaattggcaggaaaaatgcagctttcaaatcattggggggagaaaaaggatgtctttcaggattattttaattaatttttttcataattgagacagaactgtttgttatgtaccataatgctaaataaaactgtggcacttttcaccataatttaatttagtggaaaaagaagacaatgctttccatattgtgataaggtaacatggggtttttctgggccagcctttagaacactgttagggtacatacgctaccttgatgaaagggaccttcgtgcaactgtagtcatcttaaaggcttctcatccactgtgcttcttaatgtgtaattaaagtgaggagaaattaaatactctgagggcgttttatataataaattcgtgaaga

SEQ ID NO: 14 - protein, 875 aa, Homo sapiens
MEKLHQCYWKSGEPQSDDIEASRMKRAAAKHLIERYYHQLTEGCGNEACTNEFCASCPTFLRMDNNAAAIKALELYKINAKLCDPHPSKKGASSAYLENSKGAPNNSCSEIKMNKKGARIDFKDVTYLTEEKVYEILELCREREDYSPLIRVIGRVFSSAEALVQSFRKVKQHTKEELKSLQAKDEDKDEDEKEKAACSAAAMEEDSEASSSRIGDSSQGDNNLQKLGPDDVSVDIDAIRRVYTRLLSNEKIETAFLNALVYLSPNVECDLTYHNVYSRDPNYLNLFIIVMENRNLHSPEYLEMALPLFCKAMSKLPLAAQGKLIRLWSKYNADQIRRMMETFQQLITYKVISNEFNSRNLVNDDDAIVAASKCLKMVYYANVVGGEVDTNHNEEDDEEPIPESSELTLQELLGEERRNKKGPRVDPLETELGVKTLDCRKPLIPFEEFINEPLNEVLEMDKDYTFFKVETENKFSFMTCPFILNAVTKNLGLYYDNRIRMYSERRITVLYSLVQGQQLNPYLRLKVRRDHIIDDALVRLEMIAMENPADLKKQLYVEFEGEQGVDEGGVSKEFFQLVVEEIFNPDIGMFTYDESTKLFWFNPSSFETEGQFTLIGIVLGLAIYNNCILDVHFPMVVYRKLMGKKGTFRDLGDSHPVLYQSLKDLLEYEGNVEDDMMITFQISQTDLFGNPMMYDLKENGDKIPITNENRKEFVNLYSDYILNKSVEKQFKAFRRGFHMVTNESPLKYLFRPEEIELLICGSRNLDFQALEETTEYDGGYTRDSVLIREFWEIVHSFTDEQKRLFLQFTTGTDRAPVGGLGKLKMIIAKNGPDTERLPTSHTCFNVLLLPEYSSKEKLKERLLKAITYAKGFGML

SEQ ID NO: 15 - DNA, 2970 bp, Homo sapiens
tttttccggataaggaagcgcgggtcccgcatgagccccggcggtggcggcagcgaaagagaacgaggcggtggcgggcggaggcggcgggcgagggcgactacgaccagtgaggcggccgccgcagcccaggcgcgggggcgacgacaggttaaaaatctgtaagagcctgattttagaattcaccagctcctcagaagtttggcgaaatatgagttattaagcctacgctcagatcaaggtagcagctagactggtgtgacaacctgtttttaatcagtgactcaaagctgtgatcaccctgatgtcaccgaatggccacagcttgtaaaagatcaggagaacctcagtctgacgacattgaagctagccgaatgaagcgagcagctgcaaagcatctaatagaacgctactaccaccagttaactgagggctgtggaaatgaagcctgcacgaatgagttttgtgcttcctgtccaacttttcttcgtatggataataatgcagcagctattaaagccctcgagctttataagattaatgcaaaactctgtgatcctcatccctccaagaaaggagcaagctcagcttaccttgagaactcgaaaggtgcccccaacaactcctgctctgagataaaaatgaacaagaaaggcgctagaattgattttaaagatgtgacttacttaacagaagagaaggtatatgaaattcttgaattatgtagagaaagagaggattattcccctttaatccgtgttattggaagagttttttctagtgctgaggcattggtacagagcttccggaaagttaaacaacacaccaaggaagaactgaaatctcttcaagcaaaagatgaagacaaagatgaagatgaaaaggaaaaagctgcatgttctgctgctgctatggaagaagactcagaggcatcttcctcaaggataggtgatagctcacagggagacaacaatttgcaaaaattaggccctgatgatgtgtctgtggatattgatgccattagaagggtctacaccagattgctctctaatgaaaaaattgaaactgcctttctcaatgcacttgtatatttgtcacctaacgtggaatgtgacttgacgtatcacaatgtatactctcgagatcctaattatctgaatttgttcattatcgtaatggagaatagaaatctccacagtcctgaatatctggaaatggctttgccattattttgcaaagcgatgagcaagctaccccttgcagcccaaggaaaactgatcagactgtggtctaaatacaatgcagaccagattcggagaatgatggagacatttcagcaacttattacttataaagtcataagcaatgaatttaacagtcgaaatctagtgaatgatgatgatgccattgttgctgcttcgaagtgcttgaaaatggtttactatgcaaatgtagtgggaggggaagtggacacaaatcacaatgaagaagatgatgaagagcccatccctgagtccagcgagctgacacttcaggaacttttgggagaagaaagaagaaacaagaaaggtcctcgagtggaccccctggaaactgaacttggtgttaaaaccctggattgtcgaaaaccacttatcccttttgaagagtttattaatgaaccactgaatgaggttctagaaatggataaagattatacttttttcaaagtagaaacagagaacaaattctcttttatgacatgtccctttatattgaatgctgtcacaaagaatttgggattatattatgacaatagaattcgcatgtacagtgaacgaagaatcactgttctctacagcttagttcaaggacagcagttgaatccatatttgagactcaaagttagacgtgaccatatcatagatgatgcacttgtccggctagagatgatcgctatggaaaatcctgcagacttgaagaagcagttgtatgtggaatttgaaggagaacaaggagttgatgagggaggtgtttccaaagaattttttcagctggttgtggaggaaatcttcaatccagatattggtatgttcacatacgatgaatctacaaaattgttttggtttaatccatcttcttttgaaactgagggtcagtttactctgattggcatagtactgggtctggctatttacaataactgtatactggatgtacattttcccatggttgtctacaggaagctaatggggaaaaaaggaacttttcgtgacttgggagactctcacccagttctatatcagagtttaaaagatttattggagtatgaagggaatgtggaagatgacatgatgatcactttccagatatcacagacagatctttttggtaacccaatgatgtatgatctaaaggaaaatggtgataaaattccaattacaaatgaaaacaggaaggaatttgtcaatctttattctgactacattctcaataaatcagtagaaaaacagttcaaggcttttcggagaggttttcatatggtgaccaatgaatctcccttaaagtacttattcagaccagaagaaattgaattgcttatatgtggaagccggaatctagatttccaagcactagaagaaactacagaatatgacggtggctataccagggactctgttctgattagggagttctgggaaatcgttcattcatttacagatgaacagaaaagactcttcttgcagtttacaacgggcacagacagagcacctgtgggaggactaggaaaattaaagatgattatagccaaaaatggcccagacacagaaaggttacctacatctcatacttgctttaatgtgcttttacttccggaatactcaagcaaagaaaaacttaaagagagattgttgaaggccatcacgtatgccaaaggatttggcatgctgtaaaacaaaacaaaacaaaataaaacaaaaaaaaggaagg